European Patent Application EP 4 268 840 A2, published November 1, 2023. Title: PEPTIDOS PARA EL TRATAMIENTO DE INFECCIONES RESPIRATORIAS DE ORIGEN VIRAL. Applicant: CENTRO DE INGENIERIA GENETICA Y BIOTECNOLOGIA. The sequence listing filed with the application follows.

SEQUENCE LISTING (23 sequences)

SEQ ID NO: 1 - protein, 18 aa, Secuencia Artificial
  Descripción de la Secuencia Artificial: peptido sintetico
RVTQMNLNDRLASLYDKV

SEQ ID NO: 2 - protein, 18 aa, Secuencia Artificial
  Descripción de la Secuencia Artificial: peptido sintetico acetilado
  MOD_RES (1): ACETYLATION
RVTQMNLNDRLASLYDKV

SEQ ID NO: 3 - protein, 18 aa, Secuencia Artificial
  Descripción de la Secuencia Artificial: peptido sintetico acetilado y N6 es un D aminoacido
  MOD_RES (1): ACETYLATION
RVTQMNLNDRLASLYDKV

SEQ ID NO: 4 - protein, 18 aa, Secuencia Artificial
  Descripción de la Secuencia Artificial: peptido sintetico acetilado y N8 es un D aminoacido
  MOD_RES (1): ACETYLATION
RVTQMNLNDRLASLYDKV

SEQ ID NO: 5 - protein, 18 aa, Secuencia Artificial
  Descripción de la Secuencia Artificial: peptido sintetico acetilado y D9 es un D aminoacido
  MOD_RES (1): ACETYLATION
RVTQMNLNDRLASLYDKV

SEQ ID NO: 6 - protein, 18 aa, Secuencia Artificial
  Descripción de la Secuencia Artificial: peptido sintetico
RATQMNLNDRLASLYDKV

SEQ ID NO: 7 - protein, 18 aa, Secuencia Artificial
  Descripción de la Secuencia Artificial: peptido sintetico
RVTAMNLNDRLASLYDKV

SEQ ID NO: 8 - protein, 18 aa, Secuencia Artificial
  Descripción de la Secuencia Artificial: peptido sintetico
RVTQANLNDRLASLYDKV

SEQ ID NO: 9 - protein, 18 aa, Secuencia Artificial
  Descripción de la Secuencia Artificial: peptido sintetico
RVTQMNANDRLASLYDKV

SEQ ID NO: 10 - protein, 18 aa, Secuencia Artificial
  Descripción de la Secuencia Artificial: peptido sintetico
RVTQMNLNARLASLYDKV

SEQ ID NO: 11 - protein, 18 aa, Secuencia Artificial
  Descripción de la Secuencia Artificial: peptido sintetico
RVTQMNLNDRLVSLYDKV

SEQ ID NO: 12 - protein, 18 aa, Secuencia Artificial
  Descripción de la Secuencia Artificial: peptido sintetico
RVTQMNLNDRLASLYAKV

SEQ ID NO: 13 - protein, 18 aa, Secuencia Artificial
  Descripción de la Secuencia Artificial: peptido sintetico
RVTQMNLNDRLASLYDAV

SEQ ID NO: 14 - protein, 11 aa, Secuencia Artificial
  Descripción de la Secuencia Artificial: peptido sintetico
NDRLASLYDKV

SEQ ID NO: 15 - protein, 13 aa, Secuencia Artificial
  Descripción de la Secuencia Artificial: peptido sintetico
NLNDRLASLYDKV

SEQ ID NO: 16 - protein, 18 aa, Secuencia Artificial
  Descripción de la Secuencia Artificial: peptido sintetico
RVTQMNLADRLASLYDKV

SEQ ID NO: 17 - protein, 18 aa, Secuencia Artificial
  Descripción de la Secuencia Artificial: peptido sintetico
RVTQMNLNDALASLYDKV

SEQ ID NO: 18 - protein, 18 aa, Secuencia Artificial
  Descripción de la Secuencia Artificial: peptido sintetico
RVTQMNLNDRLAALYDKV

SEQ ID NO: 19 - protein, 18 aa, Secuencia Artificial
  Descripción de la Secuencia Artificial: peptido sintetico donde N6 es un D aminoacido
RVTQMNLNDRLASLYDKV

SEQ ID NO: 20 - protein, 18 aa, Secuencia Artificial
  Descripción de la Secuencia Artificial: peptido sintetico donde N8 es un D aminoacido
RVTQMNLNDRLASLYDKV

SEQ ID NO: 21 - protein, 18 aa, Secuencia Artificial
  Descripción de la Secuencia Artificial: peptido sintetico
RVTQMNLNDRAASLYDKV

SEQ ID NO: 22 - protein, 18 aa, Secuencia Artificial
  Descripción de la Secuencia Artificial: peptido sintetico
RVTQMNLNDRLASLADKV

SEQ ID NO: 23 - protein, 25 aa, Secuencia Artificial
  Descripción de la Secuencia Artificial: peptido sintetico antiviral con enlace disulfuro entre C15 y C25
GRKKRRQRRRPPQACWMSPRHLGTC